European Patent Application EP 4 159 875 A1, published April 5, 2023. Title: Novel Coronavirus Rapid Detection Kit Based on Thermal Convection PCR. Applicant: Daan Gene Co., Ltd. The sequence listing filed with the application follows.

SEQUENCE LISTING (21 sequences)

SEQ ID NO: 1 - DNA, 22 bp, Artificial sequence
  Primer
ggggaacttctcctgctagaat

SEQ ID NO: 2 - DNA, 22 bp, Artificial sequence
  Primer
cagacattttgctctcaagctg

SEQ ID NO: 3 - DNA, 20 bp, Artificial sequence
  Probe
ttgctgctgcttgacagatt

SEQ ID NO: 4 - DNA, 21 bp, Artificial sequence
  Primer
ccctgtgggttttacacttaa

SEQ ID NO: 5 - DNA, 19 bp, Artificial sequence
  Primer
acgattgtgcatcagctga

SEQ ID NO: 6 - DNA, 28 bp, Artificial sequence
  Probe
ccgtctgcggtatgtggaaaggttatgg

SEQ ID NO: 7 - DNA, 18 bp, Artificial sequence
  Primer
acacctctggatgccact

SEQ ID NO: 8 - DNA, 22 bp, Artificial sequence
  Primer
ctccgtacactctcctaccctc

SEQ ID NO: 9 - DNA, 19 bp, Artificial sequence
  Probe
ccattgccagtccgccgtc

SEQ ID NO: 10 - DNA, 19 bp, Artificial sequence
  Primer
ctaagaagcctcggcaaaa

SEQ ID NO: 11 - DNA, 17 bp, Artificial sequence
  Primer
cgtctgccgaaagcttg

SEQ ID NO: 12 - DNA, 25 bp, Artificial sequence
  Probe
ttacattgtatgctttagtggcagt

SEQ ID NO: 13 - DNA, 20 bp, Artificial sequence
  Primer
gaccccaaaatcagcgaaat

SEQ ID NO: 14 - DNA, 24 bp, Artificial sequence
  Primer
tctggttactgccagttgaatctg

SEQ ID NO: 15 - DNA, 24 bp, Artificial sequence
  Probe
accccgcattacgtttggtggacc

SEQ ID NO: 16 - DNA, 20 bp, Artificial sequence
  Primer
ttacaaacattggccgcaaa

SEQ ID NO: 17 - DNA, 18 bp, Artificial sequence
  Primer
gcgcgacattccgaagaa

SEQ ID NO: 18 - DNA, 23 bp, Artificial sequence
  Probe
acaatttgcccccagcgcttcag

SEQ ID NO: 19 - DNA, 350 bp, SARS-CoV-2
atcacgtagtcgcaacagttcaagaaattcaactccaggcagcagtaggggaacttctcctgctagaatggctggcaatggcggtgatgctgctcttgctttgctgctgcttgacagattgaaccagcttgagagcaaaatgtctggtaaaggccaacaacaacaaggccaaactgtcactaagaaatctgctgctgaggcttctaagaagcctcggcaaaaacgtactgccactaaagcatacaatgtaacacaagctttcggcagacgtggtccagaacaaacccaaggaaattttggggaccaggaactaatcagacaaggaactgattacaaacattggccgcaaa

SEQ ID NO: 20 - DNA, 350 bp, SARS-CoV-2
ggattttgtgacttaaaaggtaagtatgtacaaatacctacaacttgtgctaatgaccctgtgggttttacacttaaaaacacagtctgtaccgtctgcggtatgtggaaaggttatggctgtagttgtgatcaactccgcgaacccatgcttcagtcagctgatgcacaatcgtttttaaaccgggtttgcggtgtaagtgcagcccgtcttacaccgtgcggcacaggcactagtactgatgtcgtatacagggcttttgacatctacaatgataaagtagctggttttgctaaattcctaaaaactaattgttgtcgcttccaagaaaaggacgaagatgacaattt

SEQ ID NO: 21 - DNA, 381 bp, SARS-CoV-2
ggtgcccaccagcaggatgggcacatcagggcagtggtggcacacctctggatgccacttgtgccgcacgttctcataggacggcggactggcaatggagaaacagatgacgaaaacgttggtctgagggtaggagagtgtacggaggcggtcatactcctcctggcccgcagtgtcccacaggttcaggttcactgtgcgcccgtcaactgcgctctgcgcgctgtaattgtcgaacacggtggggatgtactctttggggaaagcgttagttgtgtagcagatgagcaggcacgtcttgcccacagccccatcacccaccaccacgcacttgatgctctgcatcgtgggtgcagttgctgtagtggaggcagtgcctcc